European Patent Application EP 4 407 033 A1, published July 31, 2024. Title: METHOD FOR PURIFYING SINGLE-STRANDED DNA. Applicant: Nanjing GenScript Biotech Co., Ltd. Application WO PCT/CN2022/127682, filed October 26, 2022. The sequence listing filed with the application follows.

SEQUENCE LISTING (18 sequences)

SEQ ID NO: 1 - DNA, 852 bp, Thermus thermophilus
  source 1..852: mol_type = genomic DNA
atgggcagcagccatcatcatcatcatcacagcagcggcctggtgccgcgcggcagccatatggctcgaggcctgaaccgcgttttcctaatcggcgccctcgccacccggccggacatgcgctacactccggcggggctcgccattttggacctgaccctcgccggtcaggacctgctcctttccgataacgggggggagcgggaggtgtcctggtaccaccgggtgaggctcttaggccgccaggcggagatgtggggcgacctcttggaccaagggcagctcgtcttcgtggagggccgcctggagtaccgccagtgggaaagggagggggagaggcggagcgagctccagatccgggccgacttcctggaccccctggacgaccgggggaaggagcgggcggaggacagccggggccagcccaggctccgcgccgccctgaaccaggtcttcctcatgggcaacctgacccgggacccggaactccgctacaccccccagggcaccgcggtggcccggctgggcctggcggtgaacgagcgccgccagggggcggaggagcgcacccacttcgtggaggttcaggcctggcgcgacctggcggagtgggccgccgagctgaggaagggcgacggccttttcgtgatcggcaggttggtgaacgactcctggaccagctccagcggcgagcggcgcttccagacccgtgtggaggccctcaggctggagcgccccacccgtggacctgcccaggccggcggaagcaggtcccgcgaagtccagacgggtggggtggacattgacgaaggcttggaagaccctccgccggaggaggagttgccgttttga

SEQ ID NO: 2 - protein, 283 aa, Thermus thermophilus
MGSSHHHHHHSSGLVPRGSHMARGLNRVFLIGALATRPDMRYTPAGLAILDLTLAGQDLLLSDNGGEREVSWYHRVRLLGRQAEMWGDLLDQGQLVFVEGRLEYRQWEREGERRSELQIRADFLDPLDDRGKERAEDSRGQPRLRAALNQVFLMGNLTRDPELRYTPQGTAVARLGLAVNERRQGAEERTHFVEVQAWRDLAEWAAELRKGDGLFVIGRLVNDSWTSSSGERRFQTRVEALRLERPTRGPAQAGGSRSREVQTGGVDIDEGLEDPPPEEELPF

SEQ ID NO: 3 - DNA, 1630 bp, synthetic construct
  source 1..1630: mol_type = other DNA
ggtttccttgagtggcaggccaggcctggccgtgaacgttcactgaaatcatggcctcttggccaagattgatagcttgtgcctgtccctgagtcccagtccatcacgagcagctggtttctaagatgctatttcccgtataaagcatgagaccgtgacttgccagccccacagagccccgcccttgtccatcactggcatctggactccagcctgggttggggcaaagagggaaatgagatcatgtcctaaccctgatcctcttgtcccacagatatccagaaccctgaccctgccgtgggaagcggagctactaacttcagcctgctgaagcaggctggagacgtggaggagaaccctggacctatggtgagcaagggcgaggagctgttcaccggggtggtgcccatcctggtcgagctggacggcgacgtaaacggccacaagttcagcgtgtccggcgagggcgagggcgatgccacctacggcaagctgaccctgaagttcatctgcaccaccggcaagctgcccgtgccctggcccaccctcgtgaccaccctgacctacggcgtgcagtgcttcagccgctaccccgaccacatgaagcagcacgacttcttcaagtccgccatgcccgaaggctacgtccaggagcgcaccatcttcttcaaggacgacggcaactacaagacccgcgccgaggtgaagttcgagggcgacaccctggtgaaccgcatcgagctgaagggcatcgacttcaaggaggacggcaacatcctggggcacaagctggagtacaactacaacagccacaacgtctatatcatggccgacaagcagaagaacggcatcaaggtgaacttcaagatccgccacaacatcgaggacggcagcgtgcagctcgccgaccactaccagcagaacacccccatcggcgacggccccgtgctgctgcccgacaaccactacctgagcacccagtccgccctgagcaaagaccccaacgagaagcgcgatcacatggtcctgctggagttcgtgaccgccgccgggatcactctcggcatggacgagctgtacaagtaatgatcataatcaagccatatcacatctgtagaggtttacttgctttaaaaaacctccacacctccccctgaacctgaaacataaaatgaatgcaattgttgttgttaacttgtttattgcagcttataatggttacaaataaagcaatagcatcacaaatttcacaaataaagcatttttttcactgcattctagttgtggtttgtccaaactcatcaatgtatcttatcatgtctggatctgcaccagctgagagactctaaatccagtgacaagtctgtctgcctattcaccgattttgattctcaaacaaatgtgtcacaaagtaaggattctgatgtgtatatcacagacaaaactgtgctagacatgaggtctatggacttcaagagcaacagtgctgtggcctggagcaacaaatctgactttgcatgtgcaaacgccttcaacaacagcattattccagaagacaccttcttccccagcccaggtaagggcagctttggtgccttcgcaggctgtttccttgcttcaggaatggcca

SEQ ID NO: 4 - DNA, 20 bp, synthetic construct
  source 1..20: mol_type = other DNA
ggtttccttgagtggcaggc

SEQ ID NO: 5 - DNA, 20 bp, synthetic construct
  source 1..20: mol_type = other DNA
tggccattcctgaagcaagg

SEQ ID NO: 6 - DNA, 24 bp, synthetic construct
  source 1..24: mol_type = other DNA
cgccagggttttcccagtcacgac

SEQ ID NO: 7 - DNA, 24 bp, synthetic construct
  source 1..24: mol_type = other DNA
agcggataacaatttcacacagga

SEQ ID NO: 8 - DNA, 4000 bp, synthetic construct
  source 1..4000: mol_type = other DNA
ggtatcagctcactcaaaggcggtaatacggttatccacagaatcaggggataacgcaggaaagaacatgtgagcaaaaggccagcaaaaggccaggaaccgtaaaaaggccgcgttgctggcgtttttccataggctccgcccccctgacgagcatcacaaaaatcgacgctcaagtcagaggtggcgaaacccgacaggactataaagataccaggcgtttccccctggaagctccctcgtgcgctctcctgttccgaccctgccgcttaccggatacctgtccgcctttctcccttcgggaagcgtggcgctttctcatagctcacgctgtaggtatctcagttcggtgtaggtcgttcgctccaagctgggctgtgtgcacgaaccccccgttcagcccgaccgctgcgccttatccggtaactatcgtcttgagtccaacccggtaagacacgacttatcgccactggcagcagccactggtaacaggattagcagagcgaggtatgtaggcggtgctacagagttcttgaagtggtggcctaactacggctacactagaagaacagtatttggtatctgcgctctgctgaagccagttaccttcggaaaaagagttggtagctcttgatccggcaaacaaaccaccgctggtagcggtggtttttttgtttgcaagcagcagattacgcgcagaaaaaaaggatctcaagaagatcctttgatcttttctacggggtctgacgctcagtggaacgaaaactcacgttaagggattttggtcatgagattatcaaaaaggatcttcacctagatccttttaaattaaaaatgaagttttaaatcaatctaaagtatatatgagtaaacttggtctgacagttaccaatgcttaatcagtgaggcacctatctcagcgatctgtctatttcgttcatccatagttgcctgactccccgtcgtgtagataactacgatacgggagggcttaccatctggccccagtgctgcaatgataccgcgagacccacgctcaccggctccagatttatcagcaataaaccagccagccggaagggccgagcgcagaagtggtcctgcaactttatccgcctccatccagtctattaattgttgccgggaagctagagtaagtagttcgccagttaatagtttgcgcaacgttgttgccattgctacaggcatcgtggtgtcacgctcgtcgtttggtatggcttcattcagctccggttcccaacgatcaaggcgagttacatgatcccccatgttgtgcaaaaaagcggttagctccttcggtcctccgatcgttgtcagaagtaagttggccgcagtgttatcactcatggttatggcagcactgcataattctcttactgtcatgccatccgtaagatgcttttctgtgactggtgagtactcaaccaagtcattctgagaatagtgtatgcggcgaccgagttgctcttgcccggcgtcaatacgggataataccgcgccacatagcagaactttaaaagtgctcatcattggaaaacgttcttcggggcgaaaactctcaaggatcttaccgctgttgagatccagttcgatgtaacccactcgtgcacccaactgatcttcagcatcttttactttcaccagcgtttctgggtgagcaaaaacaggaaggcaaaatgccgcaaaaaagggaataagggcgacacggaaatgttgaatactcatactcttcctttttcaatattattgaagcatttatcagggttattgtctcatgagcggatacatatttgaatgtatttagaaaaataaacaaataggggttccgcgcacatttccccgaaaagtgccacctgacgtcgacggatcgggagatctcccgatcccctatggtgcactctcagtacaatctgctctgatgccgcatagttaagccagtatctgctccctgcttgtgtgttggaggtcgctgagtagtgcgcgagcaaaatttaagctacaacaaggcaaggcttgaccgacaattgcatgaagaatctgcttagggttaggcgttttgcgctgcttcgcgatgtacgggccagatatacgcgttgacattgattattgactagttattaatagtaatcaattacggggtcattagttcatagcccatatatggagttccgcgttacataacttacggtaaatggcccgcctggctgaccgcccaacgacccccgcccattgacgtcaataatgacgtatgttcccatagtaacgccaatagggactttccattgacgtcaatgggtggagtatttacggtaaactgcccacttggcagtacatcaagtgtatcatatgccaagtacgccccctattgacgtcaatgacggtaaatggcccgcctggcattatgcccagtacatgaccttatgggactttcctacttggcagtacatctacgtattagtcatcgctattaccatggtgatgcggttttggcagtacatcaatgggcgtggatagcggtttgactcacggggatttccaagtctccaccccattgacgtcaatgggagtttgttttggcaccaaaatcaacgggactttccaaaatgtcgtaacaactccgccccattgacgcaaatgggcggtaggcgtgtacggtgggaggtctatataagcagagctctctggctaactagagaacccactgcttactggcttatcgaaattaatacgactcactatagggagacccaagctggctagcgtttaaacttaagcttggtaccgagctcggatccactagtccagtgtggtggaattctgcagatatccagcacagtggcggccgctcgagtctagagggcccgtttaaacccgctgatcagcctcgactgtgccttctagttgccagccatctgttgtttgcccctcccccgtgccttccttgaccctggaaggtgccactcccactgtcctttcctaataaaatgaggaaattgcatcgcattgtctgagtaggtgtcattctattctggggggtggggtggggcaggacagcaagggggaggattgggaagacaatagcaggcatgctggggatgcggtgggctctatggcttctgaggcggaaagaaccagctggggctctagggggtatccccacgcgccctgtagcggcgcattaagcgcggcgggtgtggtggttacgcgcagcgtgaccgctacacttgccagcgccctagcgcccgctcctttcgctttcttcccttcctttctcgccacgttcgccggctttccccgtcaagctctaaatcgggggctccctttagggttccgatttagtgctttacggcacctcgaccccaaaaaacttgattagggtgatggttcacgtagtgggccatcgccctgatagacggtttttcgccctttgacgttggagtccacgttctttaatagtggactcttgttccaaactggaacaacactcaaccctatctcggtctattcttttgatttataagggattttgccgatttcggcctattggttaaaaaatgagctgatttaacaaaaatttaacgcgaattaattctgtggaatgtgtgtcagttagggtgtggaaagtccccaggctccccagcaggcagaagtatgcaaagcatgcatctcaattagtcagcaaccaggtgtggaaagtccccaggctccccagcaggcagaagtatgcaaagcatgcatctcaattagtcagcaaccatagtcccgcccctaactccgcccatcccgcccctaactccgcccagttccgcccattctccgccccatggctgactaattttttttatttatgcagaggccgaggccgcctctgcctctgagctattccagaagtagtgaggaggcttttttggaggcctaggcttttgcaaaaagctcccgggagcttgtatatccattttcggatctgatcaagagacag

SEQ ID NO: 9 - protein, 283 aa, Thermus thermophilus
MGSSHHHHHHSSGLVPRGSHMARGLNRVFLIGALATRPDMRYTPAGLAILDLTLAGQDLLLSDNGGEREVSWYHRVRLLGRQAEMWGDLLDQGQLVFVEGRLEYRQWEREGERRSELQIRADFLDPLDDRGKERAEDSRGQPRLRAALNQVFLMGNLTRDPELRYTPQGTAVARLGLAVNERRQGAEERTHFVEVQAWRDLAEWAAELRKGDGLFVIGRLVNDSWTSSSGERRFQTRVEALRLERPTRGPAQAGGSRSREVQTGGVDIDEGLEDFPPEEELPF

SEQ ID NO: 10 - protein, 198 aa, Escherichia coli
MGSSHHHHHHSSGLVPRGSHMASRGVNKVILVGNLGQDPEVRYMPNGGAVANITLATSESWRDKATGEMKEQTEWHRVVLFGKLAEVASEYLRKGSQVYIEGQLRTRKWTDQSGQDRYTTEVVVNVGGTMQMLGGRQGGGAPAGGNIGGGQPQGGWGQPQQPQGGNQFSGGAQSRPQQSAPAAPSNEPPMDFDDDIPF

SEQ ID NO: 11 - protein, 142 aa, Bacillus phage Nf
MGSSHHHHHHSSGLVPRGSHMTNEIKATFDVTTLEGRMKILNAKNAGGASLKTCEDGAIIEAVGIAQYQQESDTYGDMKEETVTAIFTADGNVISAISKTVAEAASEIIDLVKEFNLDSFKVKVSKQKSSKGNEFFSLLLVG

SEQ ID NO: 12 - DNA, 20 bp, synthetic construct
  source 1..20: mol_type = other DNA
ggtatcagctcactcaaagg

SEQ ID NO: 13 - DNA, 20 bp, synthetic construct
  source 1..20: mol_type = other DNA
ctgtctcttgatcagatccg

SEQ ID NO: 14 - DNA, 20 bp, synthetic construct
  source 1..20: mol_type = other DNA
cactactcagcgacctccaa

SEQ ID NO: 15 - DNA, 20 bp, synthetic construct
  source 1..20: mol_type = other DNA
attgtctcatgagcggatac

SEQ ID NO: 16 - DNA, 20 bp, synthetic construct
  source 1..20: mol_type = other DNA
gggcaagagcaactcggtcg

SEQ ID NO: 17 - DNA, 20 bp, synthetic construct
  source 1..20: mol_type = other DNA
cctaactccgcccagttccg

SEQ ID NO: 18 - DNA, 20 bp, synthetic construct
  source 1..20: mol_type = other DNA
atagggagacccaagctggc